European Patent Application EP 4 733 387 A1, published April 29, 2026. Title: COMPOUND BACTERIAL POWDER PREPARATION, PREPARATION METHOD AND USE THEREOF. Applicant: COREE COMPANY LIMITED. The sequence listing filed with the application follows.

SEQUENCE LISTING (13 sequences)

SEQ ID NO: 1 - DNA, 1400 bp, Bifidobacterium animalis subsp. lactis HOM2120
  source 1..1400: mol_type = other DNA
  misc_feature 1..1400: note = 16S rRNA gene
tgcagtcgaacgggatccctggcagcttgctgtcggggtgagagtggcgaacgggtgagtaatgcgtgaccaacctgccctgtgcaccggaatagctcctggaaacgggtggtaataccggatgctccgctccatcgcatggtggggtgggaaatgcttttgcggcatgggatggggtcgcgtcctatcagcttgttggcggggtgatggcccaccaaggcgttgacgggtagccggcctgagagggtgaccggccacattgggactgagatacggcccagactcctacgggaggcagcagtggggaatattgcacaatgggcgcaagcctgatgcagcgacgccgcgtgcgggatggaggccttcgggttgtaaaccgcttttgttcaagggcaaggcacggtttcggccgtgttgagtggattgttcgaataagcaccggctaactacgtgccagcagccgcggtaatacgtagggtgcgagcgttatccggatttattgggcgtaaagggctcgtaggcggttcgtcgcgtccggtgtgaaagtccatcgcctaacggtggatctgcgccgggtacgggcgggctggagtgcggtaggggagactggaattcccggtgtaacggtggaatgtgtagatatcgggaagaacaccaatggcgaaggcaggtctctgggccgtcactgacgctgaggagcgaaagcgtggggagcgaacaggattagataccctggtagtccacgccgtaaacggtggatgctggatgtggggccctttccacgggtcccgtgtcggagccaacgcgttaagcatcccgcctggggagtacggccgcaaggctaaaactcaaagaaattgacgggggcccgcacaagcggcggagcatgcggattaattcgatgcaacgcgaagaaccttacctgggcttgacatgtgccggatcgccgtggagacacggtttcccttcggggccggttcacaggtggtgcatggtcgtcgtcagctcgtgtcgtgagatgttgggttaagtcccgcaacgagcgcaaccctcgccgcatgttgccagcgggtgatgccgggaactcatgtgggaccgccggggtcaactcggaggaaggtggggatgacgtcagatcatcatgccccttacgtccagggcttcacgcatgctacaatggccggtacaacgcggtgcgacacggtgacgtggggcggatcgctgaaaaccggtctcagttcggatcgcagtctgcaactcgactgcgtgaaggcggagtcgctagtaatcgcggatcagcaacgccgcggtgaatgcgttcccgggccttgtacacaccgcccgtcaagtcatgaaagtgggtagcacccgaagccggtggcccgacccttgtgggggga

SEQ ID NO: 2 - DNA, 10 bp, synthetic construct
  source 1..10: mol_type = other DNA
  misc_feature 1..10: note = OPA-02 primer
tgccgagctg

SEQ ID NO: 3 - DNA, 10 bp, synthetic construct
  source 1..10: mol_type = other DNA
  misc_feature 1..10: note = OPA-18 primer
aggtgaccgt

SEQ ID NO: 4 - DNA, 10 bp, synthetic construct
  source 1..10: mol_type = other DNA
  misc_feature 1..10: note = OPL-07 primer
aggcgggaac

SEQ ID NO: 5 - DNA, 10 bp, synthetic construct
  source 1..10: mol_type = other DNA
  misc_feature 1..10: note = OPL-16 primer
aggttgcagg

SEQ ID NO: 6 - DNA, 10 bp, synthetic construct
  source 1..10: mol_type = other DNA
  misc_structure 1..10: note = OPM-05 primer
gggaacgtgt

SEQ ID NO: 7 - DNA, 18 bp, synthetic construct
  source 1..18: mol_type = other DNA
  misc_feature 1..18: note = 27F primer
agtttgatcmtggctcag

SEQ ID NO: 8 - DNA, 19 bp, synthetic construct
  source 1..19: mol_type = other DNA
  misc_feature 1..19: note = 1492R primer
ggttaccttgttacgactt

SEQ ID NO: 9 - DNA, 891 bp, Bifidobacterium animalis subsp. lactis HOM2120
  source 1..891: mol_type = other DNA
  misc_feature 1..821: note = tuf gene
ggtatcaccatcaacattgcccacatcgagtaccagacggccaagcgtcactacgcccacgtcgactgcccgggccacgccgacttcgtgaagaacatgatcaccggcgctgcccagatggatggcgccatcctcgttgtggccgccaccgacggcccgatggcccagacccgcgagcacgtgctgctcgcccgtcaggtcggcgtcccgaagatcctcgtcgctctgaacaagtgcgatatggtcgatgacgaagagctcatcgagctcgtcgaagaagaggtccgcgacctcctcgacgagaacggcttcgaccgcgactgcccggtcgtgcacacctccgcttacggcgctctgcatgacgacgctccggatcacgacaagtgggttgccaccatcaaggagctcatggacgacgtcgacgagtacatcccgaccccggtccacgacctcgacaagccgttcctgatgccgatcgaggacgtcttcaccatctccggccgtggcaccgtcgtcaccggtcgtgtcgagcgcggcaagctgccgatcaacacgaacgtcgagatcgtcggcatccgcccgacccagaccaccaccgtcacctccatcgagaccttccacaagcagatggatgagtgcgaggccggcgacaacaccggtctgctgctccgcggcatcaaccgcaccgacgtcgagcgtggccaggtcgtggctgctccgggttcggtcaccccgcacaccaagttcgaaggcgaagtctacgtccttaccaaggatgagggcggccgtcactcgccgttcttctcgaactaccgtccgcagttctacttccgcaccaccgacgtcaccggcgtcatcacgctgccggaaggcgtcgagatggttcagcct

SEQ ID NO: 10 - DNA, 1401 bp, Bifidobacterium animalis subsp.lactis BH13-25
  source 1..1401: mol_type = other DNA
  misc_feature 1..1401: note = 16S rRNA Gene
acacatgcagtcgaacgggatccctggcagcttgctgtcggggtgagagtggcgaacgggtgagtaatgcgtgaccaacctgccctgtgcaccggaatagctcctggaaacgggtggtaataccggatgctccgctccatcgcatggtggggtgggaaatgcttttgcggcatgggatggggtcgcgtcctatcagcttgttggcggggtgatggcccaccaaggcgttgacgggtagccggcctgagagggtgaccggccacattgggactgagatacggcccagactcctacgggaggcagcagtggggaatattgcacaatgggcgcaagcctgatgcagcgacgccgcgtgcgggatggaggccttcgggttgtaaaccgcttttgttcaagggcaaggcacggtttcggccgtgttgagtggattgttcgaataagcaccggctaactacgtgccagcagccgcggtaatacgtagggtgcgagcgttatccggatttattgggcgtaaagggctcgtaggcggttcgtcgcgtccggtgtgaaagtccatcgcctaacggtggatctgcgccgggtacgggcgggctggagtgcggtaggggagactggaattcccggtgtaacggtggaatgtgtagatatcgggaagaacaccaatggcgaaggcaggtctctgggccgtcactgacgctgaggagcgaaagcgtggggagcgaacaggattagataccctggtagtccacgccgtaaacggtggatgctggatgtggggccctttccacgggtcccgtgtcggagccaacgcgttaagcatcccgcctggggagtacggccgcaaggctaaaactcaaagaaattgacgggggcccgcacaagcggcggagcatgcggattaattcgatgcaacgcgaagaaccttacctgggcttgacatgtgccggatcgccgtggagacacggtttcccttcggggccggttcacaggtggtgcatggtcgtcgtcagctcgtgtcgtgagatgttgggttaagtcccgcaacgagcgcaaccctcgccgcatgttgccagcgggtgatgccgggaactcatgtgggaccgccggggtcaactcggaggaaggtggggatgacgtcagatcatcatgccccttacgtccagggcttcacgcatgctacaatggccggtacaacgcggtgcgacacggtgacgtggggcggatcgctgaaaaccggtctcagttcggatcgcagtctgcaactcgactgcgtgaaggcggagtcgctagtaatcgcggatcagcaacgccgcggtgaatgcgttcccgggccttgtacacaccgcccgtcaagtcatgaaagtgggtagcacccgaagccggtggcccgacccttgtggg

SEQ ID NO: 11 - DNA, 1399 bp, Bifidobacterium animalis subsp.lactis BH13-33
  source 1..1399: mol_type = other DNA
  misc_feature 1..1399: note = 16S rRNA Gene
cagtcgaacgggatccctggcagcttgctgtcggggtgagagtggcgaacgggtgagtaatgcgtgaccaacctgccctgtgcaccggaatagctcctggaaacgggtggtaataccggatgctccgctccatcgcatggtggggtgggaaatgcttttgcggcatgggatggggtcgcgtcctatcagcttgttggcggggtgatggcccaccaaggcgttgacgggtagccggcctgagagggtgaccggccacattgggactgagatacggcccagactcctacgggaggcagcagtggggaatattgcacaatgggcgcaagcctgatgcagcgacgccgcgtgcgggatggaggccttcgggttgtaaaccgcttttgttcaagggcaaggcacggtttcggccgtgttgagtggattgttcgaataagcaccggctaactacgtgccagcagccgcggtaatacgtagggtgcgagcgttatccggatttattgggcgtaaagggctcgtaggcggttcgtcgcgtccggtgtgaaagtccatcgcctaacggtggatctgcgccgggtacgggcgggctggagtgcggtaggggagactggaattcccggtgtaacggtggaatgtgtagatatcgggaagaacaccaatggcgaaggcaggtctctgggccgtcactgacgctgaggagcgaaagcgtggggagcgaacaggattagataccctggtagtccacgccgtaaacggtggatgctggatgtggggccctttccacgggtcccgtgtcggagccaacgcgttaagcatcccgcctggggagtacggccgcaaggctaaaactcaaagaaattgacgggggcccgcacaagcggcggagcatgcggattaattcgatgcaacgcgaagaaccttacctgggcttgacatgtgccggatcgccgtggagacacggtttcccttcggggccggttcacaggtggtgcatggtcgtcgtcagctcgtgtcgtgagatgttgggttaagtcccgcaacgagcgcaaccctcgccgcatgttgccagcgggtgatgccgggaactcatgtgggaccgccggggtcaactcggaggaaggtggggatgacgtcagatcatcatgccccttacgtccagggcttcacgcatgctacaatggccggtacaacgcggtgcgacacggtgacgtggggcggatcgctgaaaaccggtctcagttcggatcgcagtctgcaactcgactgcgtgaaggcggagtcgctagtaatcgcggatcagcaacgccgcggtgaatgcgttcccgggccttgtacacaccgcccgtcaagtcatgaaagtgggtagcacccgaagccggtggcccgacccttgtgggggagc

SEQ ID NO: 12 - DNA, 1440 bp, Lactiplantibacillus plantarum HOM2217
  source 1..1440: mol_type = other DNA
  misc_feature 1..1440: note = 16S rRNA Gene
tatacatgcagtcgaacgaactctggtattgattggtgcttgcatcatgatttacatttgagtgagtggcgaactggtgagtaacacgtgggaaacctgcccagaagcgggggataacacctggaaacagatgctaataccgcataacaacttggaccgcatggtccgagtttgaaagatggcttcggctatcacttttggatggtcccgcggcgtattagctagatggtggggtaatggctcaccatggcaatgatacgtagccgacctgagagggtaatcggccacattgggactgagacacggcccaaactcctacgggaggcagcagtagggaatcttccacaatggacgaaagtctgatggagcaacgccgcgtgagtgaagaagggtttcggctcgtaaaactctgttgttaaagaagaacatatctgagagtaactgttcaggtattgacggtatttaaccagaaagccacggctaactacgtgccagcagccgcggtaatacgtaggtggcaagcgttgtccggatttattgggcgtaaagcgagcgcaggcggttttttaagtctgatgtgaaagccttcggctcaaccgaagaagtgcatcggaaactgggaaacttgagtgcagaagaggacagtggaactccatgtgtagcggtgaaatgcgtagatatatggaagaacaccagtggcgaaggcggctgtctggtctgtaactgacgctgaggctcgaaagtatgggtagcaaacaggattagataccctggtagtccataccgtaaacgatgaatgctaagtgttggagggtttccgcccttcagtgctgcagctaacgcattaagcattccgcctggggagtacggccgcaaggctgaaactcaaaggaattgacgggggcccgcacaagcggtggagcatgtggtttaattcgaagctacgcgaagaaccttaccaggtcttgacatactatgcaaatctaagagattagacgttcccttcggggacatggatacaggtggtgcatggttgtcgtcagctcgtgtcgtgagatgttgggttaagtcccgcaacgagcgcaacccttattatcagttgccagcattaagttgggcactctggtgagactgccggtgacaaaccggaggaaggtggggatgacgtcaaatcatcatgccccttatgacctgggctacacacgtgctacaatggatggtacaacgagttgcgaactcgcgagagtaagctaatctcttaaagccattctcagttcggattgtaggctgcaactcgcctacatgaagtcggaatcgctagtaatcgcggatcagcatgccgcggtgaatacgttcccgggccttgtacacaccgcccgtcacaccatgagagtttgtaacacccaaagtcggtggggtaaccttttaggaaccagccgc

SEQ ID NO: 13 - DNA, 452 bp, Lactiplantibacillus plantarum HOM2217
  source 1..452: mol_type = other DNA
  misc_feature 1..452: note = pheS gene
caccatattcttctggatcaatgccagacatttctaacacgtgggggtgaaccatgccggcacccagtacttcgatccaacccgtttgcttacagattgcacagcccttgccattgcaattaaagcaagttacatcagcttctacggatggttccgtgaatggaaagaagcttggccgtagccgaacatcgaattgatcgccaaacaaagtcttggcaaccagaattaaggtgcccttcaaatcagccatcgtaatatgcttgtccacgactaacccttcaatttgatgaaattgatgggaatgagttgcatcatccgtatcacgccgataaacgcggccaggtgacaagaccttcagcggtcctttagaaaaatcgtgattttcaagtgaccgcggctgatcagcagacgtctgcgtgcgtagtagcacgtctttggtaatatagaacgtg